European Patent Application EP 4 119 662 A1, published January 18, 2023. Title: PROTEIN MODIFICATION OF LIVING CELLS USING SORTASE. Applicant: Whitehead Institute for Biomedical Research. The sequence listing filed with the application follows.

SEQUENCE LISTING (138 sequences)

SEQ ID NO: 1 - protein, 206 aa, S. aureus
MKKWTNRLMTIAGVVLILVAAYLFAKPHIDNYLHDKDKDEKIEQYDKNVKEQASKDNKQQAKPQIPKDKSKVAGYIEIPDADIKEPVYPGPATPEQLNRGVSFAEENESLDDQNISIAGHTFIDRPNYQFTNLKAAKKGSMVYFKVGNETRKYKMTSIRDVKPTDVEVLDEQKGKDKQLTLITCDDYNEKTGVWEKRKIFVATEVK

SEQ ID NO: 2 - protein, 206 aa, S. aureus
MKKWTNRLMTIAGVVLILVAAYLFAKPHIDNYLHDKDKDEKIEQYDKNVKEQASKDKKQQAKPQIPKDKSKVAGYIEIPDADIKEPVYPGPATPEQLNRGVSFAEENESLDDQNISIAGHTFIDRPNYQFTNLKAAKKGSMVYFKVGNETRKYKMTSIRDVKPTDVGVLDEQKGKDKQLTLITCDDYNEKTGVWEKRKIFVATEVK

SEQ ID NO: 3 - protein, 148 aa, S. aureus
MQAKPQIPKDKSKVAGYIEIPDADIKEPVYPGPATREQLNRGVSFAEENESLDDQNISIAGHTFIDRPNYQFTNLKAAKKGSMVYFKVGNETRKYKMTSIRNVKPTAVEVLDEQKGKDKQLTLITCDDYNEETGVWETRKIFVATEVK

SEQ ID NO: 4 - protein, 148 aa, S. aureus
MQAKPQIPKDKSKVAGYIEIPDADIKEPVYPGPATREQLNRGVSFAKENQSLDDQNISIAGHTFIDRPNYQFTNLKAAKKGSMVYFKVGNETRKYKMTSIRNVKPTAVEVLDEQKGKDKQLTLITCDDYNEETGVWETRKIFVATEVK

SEQ ID NO: 5 - protein, 7 aa, Artificial Sequence
  Synthetic Polypeptide
  misc_feature (2)..(2): Xaa is Val or Ile
  misc_feature (4)..(4): Xaa can be any naturally occurring amino acid
DXEXNPG

SEQ ID NO: 6 - protein, 22 aa, Artificial Sequence
  Synthetic Polypeptide
VKQTLNFDLLKLAGDVESNPGP

SEQ ID NO: 7 - protein, 156 aa, Artificial Sequence
  Synthetic Polypeptide
MQAKPQIPKDKSKVAGYIEIPDADIKEPVYPGPATREQLNRGVSFAKENQSLDDQNISIAGHTFIDRPNYQFTNLKAAKKGSMVYFKVGNETRKYKMTSIRNVKPTAVEVLDEQKGKDKQLTLITCDDYNEETGVWETRKIFVATEVKLEHHHHHH

SEQ ID NO: 8 - protein, 5 aa, Artificial Sequence
  Synthetic Polypeptide
  misc_feature (3)..(3): Xaa can be any naturally occurring amino acid
LPXTG

SEQ ID NO: 9 - protein, 6 aa, Artificial Sequence
  Synthetic Polypeptide
  misc_feature (3)..(3): Xaa can be any naturally occurring amino acid
LPXTGG

SEQ ID NO: 10 - protein, 6 aa, Artificial Sequence
  Synthetic Polypeptide
LPETGG

SEQ ID NO: 11 - protein, 6 aa, Artificial Sequence
  Synthetic Polypeptide
  misc_feature (4)..(4): Xaa can be any naturally occurring amino acid
KLPXTG

SEQ ID NO: 12 - protein, 5 aa, Artificial Sequence
  Synthetic Polypeptide
LPETG

SEQ ID NO: 13 - protein, 8 aa, Artificial Sequence
  Synthetic Polypeptide
SIINFEKL

SEQ ID NO: 14 - protein, 5 aa, Artificial Sequence
  Synthetic Polypeptide
LPETG

SEQ ID NO: 15 - protein, 5 aa, Artificial Sequence
  Synthetic Polypeptide
LPETG

SEQ ID NO: 16 - protein, 4 aa, Artificial Sequence
  misc_feature (4)..(4): Ser can be replaced by Thr, Gly or Ala
GGGS

SEQ ID NO: 17 - protein, 5 aa, Artificial Sequence
  Synthetic Polypeptide
GGGGS

SEQ ID NO: 18 - protein, 5 aa, Artificial Sequence
  Synthetic Polypeptide
  misc_feature (2)..(2): Xaa can be any naturally occurring amino acid
LXPTG

SEQ ID NO: 19 - protein, 6 aa, Artificial Sequence
  Synthetic Polypeptide
HHHHHH

SEQ ID NO: 20-21 - skipped (2 entries)

SEQ ID NO: 22 - protein, 4 aa, Artificial Sequence
  Synthetic Polypeptide
GGGG

SEQ ID NO: 23 - protein, 5 aa, Artificial Sequence
  Synthetic Polypeptide
GGGGG

SEQ ID NO: 24 - protein, 4 aa, Artificial Sequence
  Synthetic Polypeptide
AAAA

SEQ ID NO: 25 - protein, 5 aa, Artificial Sequence
  Synthetic Polypeptide
AAAAA

SEQ ID NO: 26 - protein, 5 aa, Artificial Sequence
  Synthetic Polypeptide
LPKTG

SEQ ID NO: 27 - protein, 5 aa, Artificial Sequence
  Synthetic Polypeptide
LPATG

SEQ ID NO: 28 - protein, 5 aa, Artificial Sequence
  Synthetic Polypeptide
LPNTG

SEQ ID NO: 29 - protein, 5 aa, Artificial Sequence
  Synthetic Polypeptide
  misc_feature (3)..(3): Xaa can be any naturally occurring amino acid
LPXAG

SEQ ID NO: 30 - protein, 5 aa, Artificial Sequence
  Synthetic Polypeptide
LPNAG

SEQ ID NO: 31 - protein, 5 aa, Artificial Sequence
  Synthetic Polypeptide
  misc_feature (3)..(3): Xaa can be any naturally occurring amino acid
LPXTA

SEQ ID NO: 32 - protein, 5 aa, Artificial Sequence
  Synthetic Polypeptide
LPNTA

SEQ ID NO: 33 - protein, 5 aa, Artificial Sequence
  Synthetic Polypeptide
  misc_feature (3)..(3): Xaa can be any naturally occurring amino acid
LGXTG

SEQ ID NO: 34 - protein, 5 aa, Artificial Sequence
  Synthetic Polypeptide
LGATG

SEQ ID NO: 35 - protein, 5 aa, Artificial Sequence
  Synthetic Polypeptide
  misc_feature (3)..(3): Xaa can be any naturally occurring amino acid
IPXTG

SEQ ID NO: 36 - protein, 5 aa, Artificial Sequence
  Synthetic Polypeptide
IPNTG

SEQ ID NO: 37 - protein, 5 aa, Artificial Sequence
  Synthetic Polypeptide
IPETG

SEQ ID NO: 38 - protein, 5 aa, Artificial Sequence
  Synthetic Polypeptide
  misc_feature (3)..(3): Xaa can be any naturally occurring amino acid
TLXTC

SEQ ID NO: 39 - protein, 5 aa, Artificial Sequence
  Synthetic Polypeptide
  misc_feature (3)..(3): Xaa is Gln or Lys
  misc_feature (4)..(4): Xaa is Thr or Ser
  misc_feature (5)..(5): Xaa is Asn, Gly or Ser
NPXXX

SEQ ID NO: 40 - protein, 5 aa, Artificial Sequence
  Synthetic Polypeptide
NPQTN

SEQ ID NO: 41 - protein, 5 aa, Artificial Sequence
  Synthetic Polypeptide
NPKTG

SEQ ID NO: 42 - protein, 5 aa, Artificial Sequence
  Synthetic Polypeptide
NSKTA

SEQ ID NO: 43 - protein, 5 aa, Artificial Sequence
  Synthetic Polypeptide
NPQTG

SEQ ID NO: 44 - protein, 5 aa, Artificial Sequence
  Synthetic Polypeptide
NAKTN

SEQ ID NO: 45 - protein, 5 aa, Artificial Sequence
  Synthetic Polypeptide
NPQSS

SEQ ID NO: 46 - protein, 5 aa, Artificial Sequence
  Synthetic Polypeptide
  misc_feature (3)..(3): Xaa can be any naturally occurring amino acid
NAXTG

SEQ ID NO: 47 - protein, 5 aa, Artificial Sequence
  Synthetic Polypeptide
  misc_feature (3)..(3): Xaa can be any naturally occurring amino acid
LAXTG

SEQ ID NO: 48 - protein, 6 aa, Artificial Sequence
  Synthetic Polypeptide
QVPTGV

SEQ ID NO: 49 - protein, 5 aa, Artificial Sequence
  Synthetic Polypeptide
  misc_feature (3)..(3): Xaa can be any naturally occurring amino acid
  misc_feature (5)..(5): Xaa is Ala or Ser
LPXTX

SEQ ID NO: 50 - protein, 5 aa, Artificial Sequence
  Synthetic Polypeptide
LPSTS

SEQ ID NO: 51 - protein, 5 aa, Artificial Sequence
  Synthetic Polypeptide
  misc_feature (3)..(3): Xaa can be any naturally occurring amino acid
  misc_feature (5)..(5): Xaa can be any naturally occurring amino acid
SPXTX

SEQ ID NO: 52 - protein, 5 aa, Artificial Sequence
  Synthetic Polypeptide
  misc_feature (3)..(3): Xaa can be any naturally occurring amino acid
  misc_feature (5)..(5): Xaa can be any naturally occurring amino acid
LSXTX

SEQ ID NO: 53 - protein, 5 aa, Artificial Sequence
  Synthetic Polypeptide
  misc_feature (3)..(3): Xaa is Asp, Glu, Ala, Asn, Gln, Lys or Arg
  misc_feature (5)..(5): Xaa is Gly or Ser
NPXTX

SEQ ID NO: 54 - protein, 5 aa, Artificial Sequence
  Synthetic Polypeptide
  misc_feature (3)..(3): Xaa is Asp, Glu, Ala, Asn, Gln, Lys or Arg
  misc_feature (5)..(5): Xaa is Gly or Ser
VPXTX

SEQ ID NO: 55 - protein, 5 aa, Artificial Sequence
  Synthetic Polypeptide
  misc_feature (3)..(3): Xaa is Asp, Glu, Ala, Asn, Gln, Lys or Arg
  misc_feature (5)..(5): Xaa is Gly or Ser
IPXTX

SEQ ID NO: 56 - protein, 5 aa, Artificial Sequence
  Synthetic Polypeptide
  misc_feature (3)..(3): Xaa is Asp, Glu, Ala, Asn, Gln, Lys or Arg
  misc_feature (5)..(5): Xaa is Gly or Ser
YPXRX

SEQ ID NO: 57 - protein, 4 aa, Artificial Sequence
  Synthetic Polypeptide
LPKT

SEQ ID NO: 58 - protein, 4 aa, Artificial Sequence
  Synthetic Polypeptide
LPIT

SEQ ID NO: 59 - protein, 4 aa, Artificial Sequence
  Synthetic Polypeptide
LPDT

SEQ ID NO: 60 - protein, 4 aa, Artificial Sequence
  Synthetic Polypeptide
SPKT

SEQ ID NO: 61 - protein, 4 aa, Artificial Sequence
  Synthetic Polypeptide
LAET

SEQ ID NO: 62 - protein, 4 aa, Artificial Sequence
  Synthetic Polypeptide
LAAT

SEQ ID NO: 63 - protein, 4 aa, Artificial Sequence
  Synthetic Polypeptide
LAST

SEQ ID NO: 64 - protein, 4 aa, Artificial Sequence
  Synthetic Polypeptide
LPLT

SEQ ID NO: 65 - protein, 4 aa, Artificial Sequence
  Synthetic Polypeptide
LSRT

SEQ ID NO: 66 - protein, 4 aa, Artificial Sequence
  Synthetic Polypeptide
LPET

SEQ ID NO: 67 - protein, 4 aa, Artificial Sequence
  Synthetic Polypeptide
VPDT

SEQ ID NO: 68 - protein, 4 aa, Artificial Sequence
  Synthetic Polypeptide
IPQT

SEQ ID NO: 69 - protein, 4 aa, Artificial Sequence
  Synthetic Polypeptide
YPRR

SEQ ID NO: 70 - protein, 4 aa, Artificial Sequence
  Synthetic Polypeptide
LPMT

SEQ ID NO: 71 - protein, 4 aa, Artificial Sequence
  Synthetic Polypeptide
LAFT

SEQ ID NO: 72 - protein, 4 aa, Artificial Sequence
  Synthetic Polypeptide
LPQT

SEQ ID NO: 73 - protein, 4 aa, Artificial Sequence
  Synthetic Polypeptide
NSKT

SEQ ID NO: 74 - protein, 4 aa, Artificial Sequence
  Synthetic Polypeptide
NPQT

SEQ ID NO: 75 - protein, 4 aa, Artificial Sequence
  Synthetic Polypeptide
NAKT

SEQ ID NO: 76 - protein, 4 aa, Artificial Sequence
  Synthetic Polypeptide
NPQS

SEQ ID NO: 77 - protein, 5 aa, Artificial Sequence
  Synthetic Polypeptide
LPKTG

SEQ ID NO: 78 - protein, 5 aa, Artificial Sequence
  Synthetic Polypeptide
LPITG

SEQ ID NO: 79 - protein, 5 aa, Artificial Sequence
  Synthetic Polypeptide
LPDTA

SEQ ID NO: 80 - protein, 5 aa, Artificial Sequence
  Synthetic Polypeptide
SPKTG

SEQ ID NO: 81 - protein, 5 aa, Artificial Sequence
  Synthetic Polypeptide
LAETG

SEQ ID NO: 82 - protein, 5 aa, Artificial Sequence
  Synthetic Polypeptide
LAATG

SEQ ID NO: 83 - protein, 5 aa, Artificial Sequence
  Synthetic Polypeptide
LAHTG

SEQ ID NO: 84 - protein, 5 aa, Artificial Sequence
  Synthetic Polypeptide
LASTG

SEQ ID NO: 85 - protein, 5 aa, Artificial Sequence
  Synthetic Polypeptide
LAETG

SEQ ID NO: 86 - protein, 5 aa, Artificial Sequence
  Synthetic Polypeptide
LPLTG

SEQ ID NO: 87 - protein, 5 aa, Artificial Sequence
  Synthetic Polypeptide
LSRTG

SEQ ID NO: 88 - protein, 5 aa, Artificial Sequence
  Synthetic Polypeptide
LPETG

SEQ ID NO: 89 - protein, 5 aa, Artificial Sequence
  Synthetic Polypeptide
VPDTG

SEQ ID NO: 90 - protein, 5 aa, Artificial Sequence
  Synthetic Polypeptide
IPQTG

SEQ ID NO: 91 - protein, 5 aa, Artificial Sequence
  Synthetic Polypeptide
YPRRG

SEQ ID NO: 92 - protein, 5 aa, Artificial Sequence
  Synthetic Polypeptide
LPMTG

SEQ ID NO: 93 - protein, 5 aa, Artificial Sequence
  Synthetic Polypeptide
LPLTG

SEQ ID NO: 94 - protein, 5 aa, Artificial Sequence
  Synthetic Polypeptide
LAFTG

SEQ ID NO: 95 - protein, 5 aa, Artificial Sequence
  Synthetic Polypeptide
LPQTS

SEQ ID NO: 96 - protein, 4 aa, Artificial Sequence
  Synthetic Polypeptide
LPST

SEQ ID NO: 97 - protein, 4 aa, Artificial Sequence
  Synthetic Polypeptide
RAKR

SEQ ID NO: 98 - protein, 9 aa, Artificial Sequence
  Synthetic Polypeptide
TTCCGLRQY

SEQ ID NO: 99 - protein, 303 aa, Artificial Sequence
  Synthetic Polypeptide
IKGGLFADIASHPWQAAIFAKHHRRGGERFLCGGILISSCWILSAAHCFQQQQQEEEEERRRRRFFFFFPPPPPPHHLTVILGRTYRVVPGEEEQKFEVEKYIVHKEFDDDTYDNDIALLQLKSSSSSDDDDDSSSSSSSSSSRRRRRCAQESSVVRTVCLPPADLQLPDWTECELSGYGKHEALSPFYSERLKEAHVRLYPSSRCTTTSSSQQQHLLNRTVTDNMLCAGDTTTRRRSSSNNNLHDACQGDSGGPLVCLNDGRMTLVGIISWGLGCGGQQKDVPGVYTKVTNYLDWIRDNMRP

SEQ ID NO: 100 - protein, 255 aa, Artificial Sequence
  Synthetic Polypeptide
VVGGEDAKPGQFPWQVVLNGKVDAFCGGSIVNEKWIVTAAHCVEETTGVKITVVAGEHNIEETEHTEQKRNVIRIIPHHNYNNNAAAAAAINKYNHDIALLELDEPLVLNSYVTPICIADKEYTTTNNNIIIFLKFGSGYVSGWGRVFHKGRSALVLQYLRVPLVDRATCLRSTKFTIYNNMFCAGGFFHEGGGRRDSCQGDSGGPHVTEVEGTSFLTGIISWGEECAAMMKGKYGIYTKVSRYVNWIKEKTKLT

SEQ ID NO: 101 - protein, 57 aa, Artificial Sequence
  Synthetic Polypeptide
MTCNIKNGRCEQFCKNSADNKVVCSCTEGYRLAENQKSCEPAVPFPCGRVSVSQTSK

SEQ ID NO: 102 - protein, 496 aa, Artificial Sequence
  Synthetic Polypeptide
EFARPCIPKSFGYSSVVCVCNATYCDSFDPPALGTFSRYESTRSGRRMELSMGPIQANHTGTGLLLTLQPEQKFQKVKGFGGAMTDAAALNILALSPPAQNLLLKSYFSEEGIGYNIIRVPMASCDFSIRTYTYADTPDDFQLHNFSLPEEDTKLKIPLIHRALQLAQRPVSLLASPWTSPTWLKTNGAVNGKGSLKGQPGDIYHQTWARYFVKFLDAYAEHKLQFWAVTAENEPSAGLLSGYPFQCLGFTPEHQRDFIARDLGPTLANSTHHNVRLLMLDDQRLLLPHWAKVVLTDPEAAKYVHGIAVHWYLDFLAPAKATLGETHRLFPNTMLFASEACVGSKFWEQSVRLGSWDRGMQYSHSIITNLLYHVVGWTDWNLALNPEGGPNWVRNFVDSPIIVDITKDTFYKQPMFYHLGHFSKFIPEGSQRVGLVASQKNDLDAVALMHPDGSAVVVVLNRSSKDVPLTIKDPAVGFLETISPGYSIHTYLWHRQ

SEQ ID NO: 103 - protein, 390 aa, Artificial Sequence
  Synthetic Polypeptide
LDNGLARTPTMGWLHWERFMCNLDCQEEPDSCISEKLFMEMAELMVSEGWKDAGYEYLCIDDCWMAPQRDSEGRLQADPQRFPHGIRQLANYVHSKGLKLGIYADVGNKTCAGFPGSFGYYDIDAQTFADWGVDLLKFDGCYCDSLENLADGYKHMSLALNRTGRSIVYSCEWPLYMWPFQKPNYTEIRQYCNHWRNFADIDDSWKSIKSILDWTSFNQERIVDVAGPGGWNDPDMLVIGNFGLSWNQQVTQMALWAIMAAPLFMSNDLRHISPQAKALLQDKDVIAINQDPLGKQGYQLRQGDNFEVWERPLSGLAWAVAMINRQEIGGPRSYTIAVASLGKGVACNPACFITQLLPVKRKLGFYEWTSRLRSHINPTGTVLLQLENTM

SEQ ID NO: 104 - protein, 479 aa, Artificial Sequence
  Synthetic Polypeptide
RPPNIVLIFADDLGYGDLGCYGHPSSTTPNLDQLAAGGLRFTDFYVPVSLPSRAALLTGRLPVRMGMYPGVLVPSSRGGLPLEEVTVAEVLAARGYLTGMAGKWHLGVGPEGAFLPPHQGFHRFLGIPYSHDQGPCQNLTCFPPATPCDGGCDQGLVPIPLLANLSVEAQPPWLPGLEARYMAFAHDLMADAQRQDRPFFLYYASHHTHYPQFSGQSFAERSGRGPFGDSLMELDAAVGTLMTAIGDLGLLEETLVIFTADNGPETMRMSRGGCSGLLRCGKGTTYEGGVREPALAFWPGHIAPGVTHELASSLDLLPTLAALAGAPLPNVTLDGFDLSPLLLGTGKSPRQSLFFYPSYPDEVRGVFAVRTGKYKAHFFTQGSAHSDTTADPACHASSSLTAHEPPLLYDLSKDPGENYNLLGATPEVLQALKQLQLLKAQLDAAVTFGPSQVARGEDPALQICCHPGCTPRPACCHCP

SEQ ID NO: 105 - protein, 474 aa, Artificial Sequence
  Synthetic Polypeptide
SRPPHLVFLLADDLGWNDVGFHGSRIRTPHLDALAAGGVLLDNYYTQPLTPSRSQLLTGRYQIRTGLQHQIIWPCQPSCVPLDEKLLPQLLKEAGYTTHMVGKWHLGMYRKECLPTRRGFDTYFGYLLGSEDYYSHERCTLIDALNVTRCALDFRDGEEVATGYKNMYSTNIFTKRAIALITNHPPEKPLFLYLALQSVHEPLQVPEEYLKPYDFIQDKNRHHYAGMVSLMDEAVGNVTAALKSSGLWNNTVFIFSTDNGGQTLAGGNNWPLRGRKWSLWEGGVRGVGFVASPLLKQKGVKNRELIHISDWLPTLVKLARGHTNGTKPLDGFDVWKTISEGSPSPRIELLHNIDPNFVDSSPCSAFNTSVHAAIRHGNWKLLTGYPGCGYWFPPPSQYNVSEIPSSDPPTKTLWLFDIDRDPEERHDLSREYPHIVTKLLSRLQFYHKHSVPVYFPAQDPRCDPKATGVWGPWM

SEQ ID NO: 106 - protein, 492 aa, Artificial Sequence
  Synthetic Polypeptide
LWPWPQNFQTSDQRYVLYPNNFQFQYDVSSAAQPGCSVLDEAFQRYRDLLFGTLEKNVLVVSVVTPGCNQLPTLESVENYTLTINDDQCLLLSETVWGALRGLETFSQLVWKSAEGTFFINKTEIEDFPRFPHRGLLLDTSRHYLPLSSILDTLDVMAYNKLNVFHWHLVDDPSFPYESFTFPELMRKGSYNPVTHIYTAQDVKEVIEYARLRGIRVLAEFDTPGHTLSWGPGIPGLLTPCYSGSEPSGTFGPVNPSLNNTYEFMSTFFLEVSSVFPDFYLHLGGDEVDFTCWKSNPEIQDFMRKKGFGEDFKQLESFYIQTLLDIVSSYGKGYVVWQEVFDNKVKIQPDTIIQVWREDIPVNYMKELELVTKAGFRALLSAPWYLNRISYGPDWKDFYVVEPLAFEGTPEQKALVIGGEACMWGEYVDNTNLVPRLWPRAGAVAERLWSNKLTSDLTFAYERLSHFRCELLRRGVQAQPLNVGFCEQEFEQ

SEQ ID NO: 107 - protein, 492 aa, Artificial Sequence; identical to SEQ ID NO: 106
  Synthetic Polypeptide

SEQ ID NO: 108 - protein, 480 aa, Artificial Sequence
  Synthetic Polypeptide
PALWPLPLSVKMTPNLLHLAPENFYISHSPNSTAGPSCTLLEEAFRRYHGYIFGTQVQQLLVSITLQSECDAFPNISSDESYTLLVKEPVAVLKANRVWGALRGLETFSQLVYQDSYGTFTINESTIIDSPRFSHRGILIDTSRHYLPVKIILKTLDAMAFNKFNVLHWHIVDDQSFPYQSITFPELSNKGSYSLSHVYTPNDVRMVIEYARLRGIRVLPEFDTPGHTLSWGKGQKDLLTPCYSDSFGPINPTLNTTYSFLTTFFKEISEVFPDQFIHLGGDEVEFKCWESNPKIQDFMRQKGFGTDFKKLESFYIQKVLDIIATINKGSIVWQEVFDDKAKLAPGTIVEVWKDSAYPEELSRVTASGFPVILSAPWYLDLISYGQDWRKYYKVEPLDFGGTQKQKQLFIGGEACLWGEYVDATNLTPRLWPRASAVGERLWSSKDVRDMDDAYDRLTRHRCRMVERGIAAQPLYAGYCN

SEQ ID NO: 109 - protein, 481 aa, Artificial Sequence
  Synthetic Polypeptide
PALWPLPLSVKMTPNLLHLAPENFYISHSPNSTAGPSCTLLEEAFRRYHGYIFGTQVQQLLVSITLQSECDAFPNISSDESYTLLVKEPVAVLKANRVWGALRGLETFSQLVYQDSYGTFTINESTIIDSPRFSHRGILIDTSRHYLPVKIILKTLDAMAFNKFNVLHWHIVDDQSFPYQSITFPELSNKGSYSLSHVYTPNDVRMVIEYARLRGIRVLPEFDTPGHTLSWGKGQKDLLTPCYSLDSFGPINPTLNTTYSFLTTFFKEISEVFPDQFIHLGGDEVEFKCWESNPKIQDFMRQKGFGTDFKKLESFYIQKVLDIIATINKGSIVWQEVFDDKAKLAPGTIVEVWKDSAYPEELSRVTASGFPVILSAPWYLDLISYGQDWRKYYKVEPLDFGGTQKQKQLFIGGEACLWGEYVDATNLTPRLWPRASAVGERLWSSKDVRDMDDAYDRLTRHRCRMVERGIAAQPLYAGYCN

SEQ ID NO: 110 - protein, 492 aa, Artificial Sequence; identical to SEQ ID NO: 106
  Synthetic Polypeptide

SEQ ID NO: 111 - protein, 307 aa, Artificial Sequence
  Synthetic Polypeptide
VPWFPRTIQELDRFANQILSYGAELDADHPGFKDPVYRARRKQFADIAYNYRHGQPIPRVEYMEEEKKTWGTVFKTLKSLYKTHACYEYNHIFPLLEKYCGFHEDNIPQLEDVSQFLQTCTGFRLRPVAGLLSSRDFLGGLAFRVFHCTQYIRHGSKPMYTPEPDICHELLGHVPLFSDRSFAQFSQEIGLASLGAPDEYIEKLATIYWFTVEFGLCKQGDSIKAYGAGLLSSFGELQYCLSEKPKLLPLELEKTAIQNYTVTEFQPLYYVAESFNDAKEKVRNFAATIPRPFSVRYDPYTQRIEVL

SEQ ID NO: 112 - protein, 452 aa, Artificial Sequence
  Synthetic Polypeptide
APDQDEIQRLPGLAKQPSFRQYSGYLKSSGSKHLHYWFVESQKDPENSPVVLWLNGGPGCSSLDGLLTEHGPFLVQPDGVTLEYNPYSWNLIANVLYLESPAGVGFSYSDDKFYATNDTEVAQSNFEALQDFFRLFPEYKNNKLFLTGESYAGIYIPTLAVLVMQDPSMNLQGLAVGNGLSSYEQNDNSLVYFAYYHGLLGNRLWSSLQTHCCSQNKCNFYDNKDLECVTNLQEVARIVGNSGLNIYNLYAPCAGGVPSHFRYEKDTVVVQDLGNIFTRLPLKRMWHQALLRSGDKVRMDPPCTNTTAASTYLNNPYVRKALNIPEQLPQWDMCNFLVNLQYRRLYRSMNSQYLKLLSSQKYQILLYNGDVDMACNFMGDEWFVDSLNQKMEVQRRPWLVKYGDSGEQIAGFVKEFSHIAFLTIKGAGHMVPTDKPLAAFTMFSRFLNKQPY

SEQ ID NO: 113 - protein, 145 aa, Artificial Sequence
  Synthetic Polypeptide
LPQSFLLKCLEQVRKIQGDGAALQEKLCATYKLCHPEELVLLGHSLGIPWAPLLAGCLSQLHSGLFLYQGLLQALEGISPELGPTLDTLQLDVADFATTIWQQMEELGMMPAFASAFQRRAGGVLVASHLQSFLEVSYRVLRHLA

SEQ ID NO: 114 - protein, 105 aa, Artificial Sequence
  Synthetic Polypeptide
EHVNAIQEARRLLNLSRDTAAEMNETVEVISEMFDLQEPTCLQTRLELYKQGLRGSLTKLKGPLTMMASHYKQHCPPTPETSCATQIITFESFKENLKDFLLVIP

SEQ ID NO: 115 - protein, 165 aa, Artificial Sequence
  Synthetic Polypeptide
CDLPQTHSLGSRRTLMLLAQMRKISLFSCLKDRHDFGFPQEEFGNQFQKAETIPVLHEMIQQIFNLFSTKDSSAAWDETLLDKFYTELYQQLNDLEACVIQGVGVTETPLMKEDSILAVRKYFQRITLYLKEKKYSPCAWEVVRAEIMRSFSLSTNLQESLRSKE

SEQ ID NO: 116 - protein, 166 aa, Artificial Sequence
  Synthetic Polypeptide
MSYNLLGFLQRSSNFQCQKLLWQLNGRLEYCLKDRMNFDIPEEIKQLQQFQKEDAALTIYEMLQNIFAIFRQDSSSTGWNETIVENLLANVYHQINHLKTVLEEKLEKEDFTRGKLMSSLHLKRYYGRILHYLKAKEYSHCAWTIVRVEILRNFYFINRLTGYLRN

SEQ ID NO: 117 - protein, 242 aa, Artificial Sequence
  Synthetic Polypeptide
MQDPYVKEAENLKKYFNAGHSDVADNGTLFLGILKNWKEESDRKIMQSQIVSFYFKLFKNFKDDQSIQKSVETIKEDMNVKFFNSNKKKRDDFEKLTNYSVTDLNVQRKAIDELIQVMAELGANVSGEFVKEAENLKKYFNDNGTLFLGILKNWKEESDRKIMQSQIVSFYFKLFKNFKDDQSIQKSVETIKEDMNVKFFNSNKKKRDDFEKLTNYSVTDLNVQRKAIHELIQVMAELSPAA

SEQ ID NO: 118 - protein, 122 aa, Artificial Sequence
  Synthetic Polypeptide
STKKTQLQLEHLLLDLQMILNGINNYKNPKLTRMLTFKFYMPKKATELKHLQCLEEELKPLEEVLNLAQNFHLRPRDLISNINVIVLELKGFMCEYADETATIVEFLNRWITFCQSIISTLT

SEQ ID NO: 119 - protein, 152 aa, Artificial Sequence
  Synthetic Polypeptide
APVRSLNCTLRDSQQKSLVMSGPYELKALHLQGQDMEQQVVFSMSFVQGEESNDKIPVALGLKEKNLYLSCVLKDDKPTLQLESVDPKNYPKKKMEKRFVFNKIEINNKLEFESAQFPNWYISTSQAENMPVFLGGTKGGQDITDFTMQFVS

SEQ ID NO: 120 - protein, 148 aa, Artificial Sequence
  Synthetic Polypeptide
DKPVAHVVANPQAEGQLQWSNRRANALLANGVELRDNQLVVPIEGLFLIYSQVLFKGQGCPSTHVLLTHTISRIAVSYQTKVNLLSAIKSPCQRETPEGAEAKPWYEPIYLGGVFQLEKGDRLSAEINRPDYLDFAESGQVYFGIIAL

SEQ ID NO: 121 - protein, 144 aa, Artificial Sequence
  Synthetic Polypeptide
KPAAHLIGDPSKQNSLLWRANTDRAFLQDGFSLSNNSLLVPTSGIYFVYSQVVFSGKAYSPKATSSPLYLAHEVQLFSSQYPFHVPLLSSQKMVYPGLQEPWLHSMYHGAAFQLTQGDQLSTHTDGIPHLVLSPSTVFFGAFAL

SEQ ID NO: 122 - protein, 166 aa, Artificial Sequence
  Synthetic Polypeptide
APPRLICDSRVLERYLLEAKEAEKITTGCAEHCSLNEKITVPDTKVNFYAWKRMEVGQQAVEVWQGLALLSEAVLRGQALLVKSSQPWEPLQLHVDKAVSGLRSLTTLLRALGAQKEAISNSDAASAAPLRTITADTFRKLFRVYSNFLRGKLKLYTGEACRTGDR

SEQ ID NO: 123 - protein, 21 aa, Artificial Sequence
  Synthetic Polypeptide
GIVEQCCTSICSLYQLENYCN

SEQ ID NO: 124 - protein, 29 aa, Artificial Sequence
  Synthetic Polypeptide
FVNQHLCGSHLVEALYLVCGERGFFYTPK

SEQ ID NO: 125 - protein, 166 aa, Artificial Sequence
  Synthetic Polypeptide
FPTIPLSRLADNAWLRADRLNQLAFDTYQEFEEAYIPKEQIHSFWWNPQTSLCPSESIPTPSNKEETQQKSNLELLRISLLLIQSWLEPVQFLRSVFANSLVYGASDSNVYDLLKDLEEGIQTLMGRLEALLKNYGLLYCFNKDMSKVSTYLRTVQCRSVEGSCGF

SEQ ID NO: 126 - protein, 242 aa, Artificial Sequence
  Synthetic Polypeptide
CHHRICHCSNRVFLCQESKVTEIPSDLPRNAIELRFVLTKLRVIQKGAFSGFGDLEKIEISQNDVLEVIEADVFSNLPKLHEIRIEKANNLLYINPEAFQNLPNLQYLLISNTGIKHLPDVHKIHSLQKVLLDIQDNINIHTIERNSFVGLSFESVILWLNKNGIQEIHNCAFNGTQLDELNLSDNNNLEELPNDVFHGASGPVILDISRTRIHSLPSYGLENLKKLRARSTYNLKKLPTLE

SEQ ID NO: 127 - protein, 130 aa, Artificial Sequence
  Synthetic Polypeptide
IQKVQDDTKTLIKTIVTRINDILDFIPGLHPILTLSKMDQTLAVYQQILTSMPSRNVIQISNDLENLRDLLHVLAFSKSCHLPEASGLETLDSLGGVLEASGYSTEVVALSRLQGSLQDMLWQLDLSPGC

SEQ ID NO: 128 - protein, 62 aa, Artificial Sequence
  Synthetic Polypeptide
PETLCGAELVDALQFVCGDRGFYFNKPTGYGSSSRRAPQTGIVDECCFRSCDLRRLEMYCAP

SEQ ID NO: 129 - protein, 125 aa, Artificial Sequence
  Synthetic Polypeptide
MYRSAFSVGLETRVTVPNVPIRFTKIFYNQQNHYDGSTGKFYCNIPGLYYFSYHITVYMKDVKVSLFKKDKAVLFTYDQYQENVDQASGSVLLHLEVGDQVWLQVYYADNVNDSTFTGFLLYHDT

SEQ ID NO: 130 - protein, 111 aa, Artificial Sequence
  Synthetic Polypeptide
MYRSAFSVGLPNVPIRFTKIFYNQQNHYDGSTGKFYCNIPGLYYFSYHITVYMKDVKVSLFKKDKVLFTYDQYQEKVDQASGSVLLHLEVGDQVWLQVYDSTFTGFLLYHD

SEQ ID NO: 131 - protein, 102 aa, Artificial Sequence
  Synthetic Polypeptide
MYRSAFSVGLETRVTVPIRFTKIFYNQQNHYDGSTGKFYCNIPGLYYFSYHITVDVKVSLFKKDKAVLFTQASGSVLLHLEVGDQVWLQNDSTFTGFLLYHD

SEQ ID NO: 132 - protein, 693 aa, Artificial Sequence
  Synthetic Polypeptide
ATRRYYLGAVELSWDYMQSDLGELPVDARFPPRVPKSFPFNTSVVYKKTLFVEFTDHLFNIAKPRPPWMGLLGPTIQAEVYDTVVITLKNMASHPVSLHAVGVSYWKASEGAEYDDQTSQREKEDDKVFPGGSHTYVWQVLKENGPMASDPLCLTYSYLSHVDLVKDLNSGLIGALLVCREGSLAKEKTQTLHKFILLFAVFDEGKSWHSETKNAASARAWPKMHTVNGYVNRSLPGLIGCHRKSVYWHVIGMGTTPEVHSIFLEGHTFLVRNHRQASLEISPITFLTAQTLLMDLGQFLLFCHISSHQHDGMEAYVKVDSCPEEPQFDDDNSPSFIQIRSVAKKHPKTWVHYIAAEEEDWDYAPLVLAPDDRSYKSQYLNNGPQRIGRKYKKVRFMAYTDETFKTREAIQHESGILGPLLYGEVGDTLLIIFKNQASRPYNIYPHGITDVRPLYSRRLPKGVKHLKDFPILPGEIFKYKWTVTVEDGPTKSDPRCLTRYYSSFVNMERDLASGLIGPLLICYKESVDQRGNQIMSDKRNVILFSVFDENRSWYLTENIQRFLPNPAGVQLEDPEFQASNIMHSINGYVFDSLQLSVCLHEVAYWYILSIGAQTDFLSVFFSGYTFKHKMVYEDTLTLFPFSGETVFMSMENPGLWILGCHNSDFRNRGMTALLKVSSCDKNTGDYYEDSYED

SEQ ID NO: 133 - protein, 644 aa, Artificial Sequence
  Synthetic Polypeptide
RSFQKKTRHYFIAAVERLWDYGMSSSPHVLRNRAQSGSVPQFKKVVFQEFTDGSFTQPLYRGELNEHLGLLGPYIRAEVEDNIMVTFRNQASRPYSFYSSLISYEEDQRQGAEPRKNFVKPNETKTYFWKVQHHMAPTKDEFDCKAWAYSSDVDLEKDVHSGLIGPLLVCHTNTLNPAHGRQVTVQEFALFFTIFDETKSWYFTENMERNCRAPCNIQMEDPTFKENYRFHAINGYIMDTLPGLVMAQDQRIRWYLLSMGSNENIHSIHFSGHVFTVRKKEEYKMALYNLYPGVFETVEMLPSKAGIWRVECLIGEHLHAGMSTLFLVYSNKCQTPLGMASGHIRDFQITASGQYGQWAPKLARLHYSGSINAWSTKEPFSWIKVDLLAPMIIHGIKTQGARQKFSSLYISQFIIMYSLDGKKWQTYRGNSTGTLMVFFGNVDSSGIKHNIFNPPIIARYIRLHPTHYSIRSTLRMELMGCDLNSCSMPLGMESKAISDAQITASSYFTNMFATWSPSKARLHLQGRSNAWRPQVNNPKEWLQVDFQKTMKVTGVTTQGVKSLLTSMYVKEFLISSSQDGHQWTLFFQNGKVKVFQGNQDSFTPVVNSLDPPLLTRYLRIHPQSWVHQIALRMEVLGCEAQDLY

SEQ ID NO: 134 - protein, 578 aa, Artificial Sequence
  Synthetic Polypeptide
SEVAHRFKDLGEENFKALVLIAFAQYLQQCPFEDHVKLVNEVTEFAKTCVADESAENCDKSLHTLFGDKLCTVATLRETYGEMADCCAKQEPERNECFLQHKDDNPNLPRLVRPEVDVMCTAFHDNEETFLKKYLYEIARRHPYFYAPELLFFAKRYKAAFTECCQAADKAACLLPKLDELRDEGKASSAKQRLKCASLQKFGERAFKAWAVARLSQRFPKAEFAEVSKLVTDLTKVHTECCHGDLLECADDRADLAKYICENQDSISSKLKECCEKPLLEKSHCIAEVENDEMPADLPSLAADFVESKDVCKNYAEAKDVFLGMFLYEYARRHPDYSVVLLLRLAKTYETTLEKCCAAADPHECYAKVFDEFKPLVEEPQNLIKQNCELFEQLGEYKFQNALLVRYTKKVPQVSTPTLVEVSRNLGKVGSKCCKHPEAKRMPCAEDYLSVVLNQLCVLHEKTPVSDRVTKCCTESLVNRRPCFSALEVDETYVPKEFNAETFTFHADICTLSEKERQIKKQTALVELVKHKPKATKEQLKAVMDDFAAFVEKCCKADDKETCFAEEGKKLVAASQAA

SEQ ID NO: 135 - protein, 578 aa, Artificial Sequence; identical to SEQ ID NO: 134
  Synthetic Polypeptide

SEQ ID NO: 136 - protein, 141 aa, Artificial Sequence
  Synthetic Polypeptide
VLSPADKTNVKAAWGKVGAHAGEYGAEALERMFLSFPTTKTYFPHFDLSHGSAQVKGHGKKVADALTNAVAHVDDMPNALSALSDLHAHKLRVDPVNFKLLSHCLLVTLAAHLPAEFTPAVHASLDKFLASVSTVLTSKYR

SEQ ID NO: 137 - protein, 146 aa, Artificial Sequence
  Synthetic Polypeptide
VHLTPEEKSAVTALWGKVNVDEVGGEALGRLLVVYPWTQRFFESFGDLSTPDAVMGNPKVKAHGKKVLGAFSDGLAHLDNLKGTFATLSELHCDKLHVDPENFRLLGNVLVCVLAHHFGKEFTPPVQAAYQKVVAGVANALAHKYH

SEQ ID NO: 138 - protein, 7 aa, Artificial Sequence
  Synthetic Polypeptide
HALPETG